European Patent Specification EP 2 481 078 B1, published June 21, 2023. Title: Procédé de détection des molécules par spectrométrie de masse. Applicant: bioMérieux Université Claude Bernard Lyon 1 Centre National de la Recherche Scientifique. The sequence listing filed with the application follows.

SEQUENCE LISTING (6 sequences)

SEQ ID NO: 1 - protein, 141 aa, artificial sequence
  Protéine recombinante TP171 de Treponema pallidum
MRGSASFSSIPNGTYRATYQDFDENGWKDFLEVTFDGGKMVQVVYDYQHKEGRFKSQDADYHRVMYASSGIGPEKAFRELADALLEKGNPEMVDVVTGATVSSQSFRRLGAALLQSARRGEKEAIISRGSSKYKYHHHHHH

SEQ ID NO: 2 - protein, 9 aa, artificial sequence
  Ion protéotypique
ELADALLEK

SEQ ID NO: 3 - protein, 11 aa, artificial sequence
  Ion protéotypique
DFLEVTFDGGK

SEQ ID NO: 4 - protein, 6 aa, artificial sequence
  Ion protéotypique
EAIISR

SEQ ID NO: 5 - protein, 11 aa, artificial sequence
  Ion protéotypique
MVQVVYDYQHK

SEQ ID NO: 6 - protein, 12 aa, artificial sequence
  Peptide du PSA
LSEPAELTDAVK